European Patent Application EP 4 631 491 A1, published October 15, 2025. Title: Peptide having activities of skin condition improvement and uses thereof. Applicant: CAREGEN CO., LTD. The sequence listing filed with the application follows.

SEQUENCE LISTING (16 sequences)

SEQ ID NO: 1 - protein, 6 aa, synthetic construct
GPRGDP

SEQ ID NO: 2 - protein, 9 aa, synthetic construct
LGPRGDPGL

SEQ ID NO: 3 - protein, 9 aa, synthetic construct
SGPRGDPGL

SEQ ID NO: 4 - protein, 8 aa, synthetic construct
GPRGDPGL

SEQ ID NO: 5 - DNA, 20 bp, synthetic construct
  source 1..20: mol_type = other DNA
caccctcaagagcctgagtc

SEQ ID NO: 6 - DNA, 20 bp, synthetic construct
  source 1..20: mol_type = other DNA
agacggctgagtagggaaca

SEQ ID NO: 7 - DNA, 20 bp, synthetic construct
  source 1..20: mol_type = other DNA
ccaggaaccgagtacaccat

SEQ ID NO: 8 - DNA, 20 bp, synthetic construct
  source 1..20: mol_type = other DNA
atacccaggttgggtgatga

SEQ ID NO: 9 - DNA, 20 bp, synthetic construct
  source 1..20: mol_type = other DNA
gcaagacctggctttggact

SEQ ID NO: 10 - DNA, 21 bp, synthetic construct
  source 1..21: mol_type = other DNA
gggagtttctggttagggctg

SEQ ID NO: 11 - DNA, 20 bp, synthetic construct
  source 1..20: mol_type = other DNA
ggagccaaaagggtcatcat

SEQ ID NO: 12 - DNA, 20 bp, synthetic construct
  source 1..20: mol_type = other DNA
gtgatggcatggactgtggt

SEQ ID NO: 13 - DNA, 20 bp, synthetic construct
  source 1..20: mol_type = other DNA
tcagtggctggaacagtgag

SEQ ID NO: 14 - DNA, 20 bp, synthetic construct
  source 1..20: mol_type = other DNA
tctggcatgtcccactatca

SEQ ID NO: 15 - DNA, 20 bp, synthetic construct
  source 1..20: mol_type = other DNA
ccttcttgggtgctggaata

SEQ ID NO: 16 - DNA, 20 bp, synthetic construct
  source 1..20: mol_type = other DNA
acacgataagggaggctgtg